European Patent Specification EP 3 368 548 B1, published August 23, 2023. Title: METHANOL DEHYDROGENASE FUSION PROTEINS. Applicant: Genomatica Li, Jingyi Barton, Nelson R. Warner, Joseph R. Pharkya, Priti. The sequence listing filed with the application follows.

SEQUENCE LISTING (12 sequences)

SEQ ID NO: 1 - protein, 382 aa, Bacillus methanolicus MGA3
MTTNFFIPPASVIGRGAVKEVGTRLKQIGAKKALIVTDAFLHSTGLSEEVAKNIREAGVDVAIFPKAQPDPADTQVHEGVDVFKQENCDSLVSIGGGSSHDTAKAIGLVAANGGRINDYQGVNSVEKPVVPVVAITTTAGTGSETTSLAVITDSARKVKMPVIDEKITPTVAIVDPELMVKKPAGLTIATGMDALSHAIEAYVAKGATPVTDAFAIQAMKLINEYLPKAVANGEDIEAREKMAYAQYMAGVAFNNGGLGLVHSISHQVGGVYKLQHGICNSVNMPHVCAFNLIAKTERFAHIAELLGENVAGLSTAAAAERAIVALERINKSFGIPSGYAEMGVKEEDIELLAKNAYEDVCTQSNPRVPTVQDIAQIIKNAM

SEQ ID NO: 2 - DNA, 1149 bp, Bacillus methanolicus MGA3
atgacaacaaactttttcattccaccagccagcgtaattggacgcggtgcagtaaaggaagtaggaacaagacttaagcaaattggagctaagaaagcgcttatcgttacagatgcattccttcacagcacaggtttatctgaagaagttgctaaaaacattcgtgaagctggcgttgatgttgcgattttcccaaaagctcaaccagatccagcagatacacaagttcatgaaggtgtagatgtattcaaacaagaaaactgtgattcacttgtttctatcggtggaggtagctctcacgatacagctaaagcaatcggtttagttgcagcaaacggcggaagaatcaatgactatcaaggtgtaaacagcgtagaaaaaccagtcgttccagtagttgcaatcactacaacagctggtactggtagtgaaacaacatctcttgcggttattacagactctgcacgtaaagtaaaaatgcctgttattgatgagaaaattactccaactgtagcaattgttgacccagaattaatggtgaaaaaaccagctggattaacaatcgcaactggtatggatgcattgtcccatgcaattgaagcatatgttgcaaaaggtgctacaccagttactgatgcatttgctattcaagcaatgaaacttatcaatgaatacttaccaaaagcggttgcgaacggagaagacatcgaagcacgtgaaaaaatggcttatgcacaatacatggcaggagtggcatttaacaacggtggtttaggactagttcactctatttctcaccaagtaggtggagtttacaaattacaacacggaatctgtaactcagttaatatgccacacgtttgcgcattcaacctaattgctaaaactgagcgcttcgcacacattgctgagcttttaggtgagaatgttgctggcttaagcactgcagcagctgctgagagagcaattgtagctcttgaaagaatcaacaaatccttcggtatcccatctggctatgcagaaatgggcgtgaaagaagaggatatcgaattattagcgaaaaacgcatacgaagacgtatgtactcaaagcaacccacgcgttcctactgttcaagacattgcacaaatcatcaaaaacgctatgtaa

SEQ ID NO: 3 - protein, 211 aa, Bacillus methanolicus MGA3
MELQLALDLVNIEEAKQVVAEVQEYVDIVEIGTPVIKIWGLQAVKAVKDAFPHLQVLADMKTMDAAAYEVAKAAEHGADIVTILAAAEDVSIKGAVEEAKKLGKKILVDMIAVKNLEERAKQVDEMGVDYICVHAGYDLQAVGKNPLDDLKRIKAVVKNAKTAIAGGIKLETLPEVIKAEPDLVIVGGGIANQTDKKAAAEKINKLVKQGL

SEQ ID NO: 4 - protein, 184 aa, Bacillus methanolicus MGA3
MLTTEFLAEIVKELNSSVNQIADEEAEALVNGILQSKKVFVAGAGRSGFMAKSFAMRMMHMGIDAYVVGETVTPNYEKEDILIIGSGSGETKSLVSMAQKAKSIGGTIAAVTINPESTIGQLADIVIKMPGSPKDKSEARETIQPMGSLFEQTLLLFYDAVILRFMEKKGLDTKTMYGRHANLE

SEQ ID NO: 5 - protein, 406 aa, Artificial Sequence
  fusion protein
MKLQVAIDLLSTEAALELAGKVAEYVDIIELGTPLIKAEGLSVITAVKKAHPDKIVFADMKTMDAGELEADIAFKAGADLVTVLGSADDSTIAGAVKAAQAHNKGVVVDLIGIEDKATRAQEVRALGAKFVEMHAGLDEQAKPGFDLNGLLAAGEKARVPFSVAGGVKVATIPAVQKAGAEVAVAGGAIYGAADPAAAAKELRAAIAMTQAAEADGAVKVVGDDITNNLSLVRDEVADTAAKVDPEQVAVLARQIVQPGRVFVAGAGRSGLVLRMAAMRLMHFGLTVHVAGDTTTPAISAGDLLLVASGSGTTSGVVKSAETAKKAGARIAAFTTNPDSPLAGLADAVVIIPAAQKTDHGSHISRQYAGSLFEQVLFVVTEAVFQSLWDHTEVEAEELWTRHANLE

SEQ ID NO: 6 - protein, 388 aa, Desulfotomaculum reducens MI-1
MTVGEQVFGYFIPTVNLMGVGAHKEIPDQVKVLGGSNVLIVTDAFLGRPGGMADDIKGMLEAENIKVTIYAGAEPNPTDVNVHDGLKVYQECGADMILSLGGGSSHDCAKGIGIVATNGGNIRDYEGINKSSKAMPPFIAVNTTAGTASEMTRFCIITNTSNHVKMAIVDWRCTPNIAINDPLLMAGMPPALTAATGMDALTHAIEAYVSVAATPVTDSAALMAIKLISQYLRAAVANGENMEARDKMAYAEFLGGMAFNNASLGYVHAMAHQLGGFYNLPHGVCNAILLPHVEAFNLIACPERFVDIAVAMGENVEGLSVRDAADKALSAIRKLSADVGIPAGLTELGVKEEDLKTMAENAMKDACALTNPRKATLNDIVGIYKTAL

SEQ ID NO: 7 - protein, 20 aa, Artificial Sequence
  linker sequence
GGSGGSGSGSGGSGSGSGGS

SEQ ID NO: 8 - protein, 382 aa, Artificial Sequence
  MeDH variant
MTTNFFIPPASVIGRGAVKEVGTRLKQIGAKKALIVTDAFLHSTGLSEEVAKNIREAGVDVAIFPKAQPDPADTQVHEGVDVFKQENCDSLVSIGGGSSHDTAKAIGLVAANGGRINDYQGVNSVEKPMIPVVAITTTAGTGSETTSLAVITDSARKVKMPVIDEKITPTVAIVDPELMVKKPAGLTIATGMDALSHAIEAYVAKGATPVTDAFAIQAMKLINEYLPKAVANGEDIEAREKMAYAQYMAGVAFNNGGLGLVHSISHQVGSVYKLQHGICNSVNMPHVCAFNLIAKTERFAHIAELLGENVAGLSTAAAAERAIVALERINKSFGIPSGYAEMGVKEEDIELLAKDAYEDVCTQSNPRVPTVQDIAQIIKNAM

SEQ ID NO: 9 - DNA, 1149 bp, Artificial Sequence
  MeDH variant
atgaccaccaactttttcatcccaccagcatcagttatcggtagaggcgcagttaaagaagttggcacccgtctgaagcaaatcggtgcgaagaaagctctgattgttaccgacgcgtttctgcatagcaccggtttgagcgaagaagtggcgaagaacattcgtgaagcgggcgtcgatgtggcgattttcccgaaagcccagccggaccctgccgatacgcaagtccacgaaggtgttgatgtctttaaacaggagaattgcgacagcttggttagcatcggtggcggctcttcccatgatacggcgaaagcaattggcctggtcgcagcaaatggtggccgtatcaatgactaccagggtgttaacagcgtggagaagccgatgattccggtggtcgcgatcacgactacggcaggcaccggctccgaaaccaccagcttggcggtcatcacggatagcgcgcgtaaagtgaaaatgccggtgatcgatgagaaaatcaccccgaccgtggcgattgtcgatccggagctgatggtgaagaagccggctggtttgaccattgcaaccggtatggacgccctgtctcacgccatcgaagcatacgtggcaaagggtgcgacgccggtgaccgatgcgttcgccattcaggcaatgaaactgattaatgagtatctgccgaaggctgttgcgaatggcgaggacatcgaggcacgcgagaaaatggcgtatgctcaatacatggccggtgtcgcgttcaacaatggtggtctgggtctggtacacagcatcagccaccaagtgggtagtgtgtacaaactgcaacacggcatttgcaactccgtcaacatgccgcacgtttgtgcgtttaatctgattgccaagaccgaacgtttcgcccatatcgctgagctgctgggtgagaacgttgcaggcctgagcacggcggctgcggcggagcgcgcaattgtcgcgctggaacgcattaacaagagctttggtatcccgagcggctatgcggagatgggtgtgaaagaagaggacattgaactgctggctaaggatgcgtacgaggacgtttgtactcagagcaacccgcgtgttccgacggtccaggacattgcccagattatcaagaacgcgatgtag

SEQ ID NO: 10 - protein, 393 aa, uncultured organism
MSLVNYLQLADRTDGFFIPSVTLVGPGCVKEVGPRAKMLGAKRALIVTDAGLHKMGLSQEIADLLRSEGIDSVIFAGAEPNPTDINVHDGVKVYQKEKCDFIVSLGGGSSHDCAKGIGLVTAGGGHIRDYEGVDKSKVPMTPLIAINTTAGTASEMTRFCIITNTDTHVKMAIVDWRCTPLVAIDDPRLMVKMPPALTAATGMDALTHAVEAYVSTAATPITDTCAEKAIELIGQWLPKAVANGDWMEARAAMCYAQYLAGMAFNNASLGYVHAMAHQLGGFYNLPHGVCNAILLPHVCQFNLIAATERYARIAALLGVDTSGMETREAALAAIAAIKELSSSIGIPRGLSELGVKAADHKVMAENAQKDACMLTNPRKATLEQVIGIFEAAM

SEQ ID NO: 11 - DNA, 1182 bp, uncultured organism
atgagcctggttaattatctgcagctggccgatcgtaccgatggcttttttatcccgagcgttaccctggttggtccgggttgtgttaaagaagttggtcctcgcgcaaaaatgctgggtgcaaaacgtgcactgattgttaccgatgcaggtctgcacaaaatgggtctgagccaagaaattgccgatctgctgcgtagcgaaggtattgatagcgttatttttgccggtgcagaaccgaatccgaccgatatcaatgttcatgatggtgtgaaagtgtatcagaaagagaaatgcgattttatcgttagcctgggtggtggtagcagccatgattgtgcaaaaggtattggtctggttaccgcaggcggtggtcatattcgtgattatgaaggtgttgacaaaagcaaagttccgatgacaccgctgattgcaattaataccaccgcaggcaccgcaagcgaaatgacccgtttttgtattattaccaacaccgatacccatgtgaaaatggcaattgttgattggcgttgtactccgctggttgccattgatgatccgcgtctgatggttaaaatgcctccggcactgaccgcagcaaccggtatggatgcactgacccatgcagttgaagcatatgtgagcaccgcagccaccccgattaccgatacctgtgcagaaaaagcaattgaactgattggtcagtggctgccgaaagcagttgcaaatggtgattggatggaagcacgtgcagcaatgtgttatgcacagtatctggcaggtatggcattcaataatgcaagcctgggttatgttcatgcaatggcacatcagctgggtggcttttataacctgccgcatggtgtttgtaatgcaattctgctgcctcatgtttgccagtttaatctgattgcagccaccgaacgttatgcccgtattgcagcactgctgggtgttgataccagcggtatggaaacccgtgaagcagcactggcagcaattgccgcaattaaagaactgagcagcagcattggtattccgcgtggtctgagcgaactgggtgttaaagcagccgatcataaagttatggcagaaaatgcacagaaagatgcatgtatgctgacaaatccgcgtaaagcaaccctggaacaggttattggtatttttgaagccgcaatgtag

SEQ ID NO: 12 - protein, 185 aa, Bacillus methanolicus
MGKLFEEKTIKTEQIFSGRVVKLQVDDVELPNGQTSKREIVRHPGAVAVIAITNENKIVMVEQYRKPLEKSIVEIPAGKLEKGEDPRITALRELEEETGYECEQMEWLISFATSPGFADEIIHIYVAKGLSKKENAAGLDEDEFVDLIELTLDEALQYIKEQRIYDSKTVIAVQYLQLQEALKNK